European Patent Application EP 4 342 980 A1, published March 27, 2024. Title: Production method of brain microvascular endothelial-like cells and use thereof. Applicant: PUBLIC UNIVERSITY CORPORATION NAGOYA CITY UNIVERSITY. The sequence listing filed with the application follows.

SEQUENCE LISTING (24 sequences)

SEQ ID NO: 1 - DNA, 20 bp, Artificial Sequence
  CDH5 forward primer
gatttggaaccagatgcaca

SEQ ID NO: 2 - DNA, 20 bp, Artificial Sequence
  CDH5 reverse primer
acttggcattcttgcgactc

SEQ ID NO: 3 - DNA, 20 bp, Artificial Sequence
  MDR1 forward primer
cccatcattgcaatagcagg

SEQ ID NO: 4 - DNA, 21 bp, Artificial Sequence
  MDR1 reverse primer
tgttcaaacttctgctcctga

SEQ ID NO: 5 - DNA, 22 bp, Artificial Sequence
  BCRP forward primer
agatgggtttccaagcgttcat

SEQ ID NO: 6 - DNA, 23 bp, Artificial Sequence
  BCRP reverse primer
ccagtcccagtacgactgtgaca

SEQ ID NO: 7 - DNA, 21 bp, Artificial Sequence
  GLUT1 forward primer
gaagagagtcggcagatgatg

SEQ ID NO: 8 - DNA, 25 bp, Artificial Sequence
  GLUT1 reverse primer
ggagtaatagaagacagcgttgatg

SEQ ID NO: 9 - DNA, 20 bp, Artificial Sequence
  Occludin forward primer
tccaatggcaaagtgaatga

SEQ ID NO: 10 - DNA, 20 bp, Artificial Sequence
  Occludin reverse primer
gcaggtgctctttttgaagg

SEQ ID NO: 11 - DNA, 23 bp, Artificial Sequence
  ZO-1 forward primer
cgagggatagaagtgcaagtaga

SEQ ID NO: 12 - DNA, 23 bp, Artificial Sequence
  ZO-1 reverse primer
tattcttcatttttccgggattt

SEQ ID NO: 13 - DNA, 20 bp, Artificial Sequence
  LAT1 forward primer
aatgggtccctgttcacatc

SEQ ID NO: 14 - DNA, 20 bp, Artificial Sequence
  LAT1 reverse primer
cgtagagcagcgtcatcaca

SEQ ID NO: 15 - DNA, 20 bp, Artificial Sequence
  HPRT1 forward primer
ctttgctttccttggtcagg

SEQ ID NO: 16 - DNA, 21 bp, Artificial Sequence
  HPRT1 reverse primer
tcaagggcatatcctacaaca

SEQ ID NO: 17 - DNA, 20 bp, Artificial Sequence
  PECAM1 forward primer
agtcggacagtgggacgtat

SEQ ID NO: 18 - DNA, 20 bp, Artificial Sequence
  PECAM1 reverse primer
atgacctcaaactgggcatc

SEQ ID NO: 19 - DNA, 20 bp, Artificial Sequence
  PDGFR-beta forward primer
tcagagctgacactggttcg

SEQ ID NO: 20 - DNA, 20 bp, Artificial Sequence
  PDGFR-beta reverse primer
cagggtggctctcacttagc

SEQ ID NO: 21 - DNA, 23 bp, Artificial Sequence
  NG2 forward primer
ctacaagtgaccattgccctaga

SEQ ID NO: 22 - DNA, 24 bp, Artificial Sequence
  NG2 reverse primer
gctcttcactgagaatacgatgtc

SEQ ID NO: 23 - DNA, 20 bp, Artificial Sequence
  alpha-SMA forward primer
gcctgagggaaggtcctaac

SEQ ID NO: 24 - DNA, 20 bp, Artificial Sequence
  alpha-SMA reverse primer
cagagccattgtcacacacc